European Patent Specification EP 3 294 893 B1, published December 27, 2023. Title: BIO-PRODUCTION OF LENTIVIRAL VECTORS. Applicant: LEE, Chi-Lin BARTLETT, Jeffrey. The sequence listing filed with the application follows.

SEQUENCE LISTING (15 sequences)

SEQ ID NO: 1 - DNA, 6565 bp, Artificial Sequence
  Synthetic: PUC57-TL20C
ggccgcctcggccaaacagcccttgagtttaccactccctatcagtgatagagaaaagtgaaagtcgagtttaccactccctatcagtgatagagaaaagtgaaagtcgagtttaccactccctatcagtgatagagaaaagtgaaagtcgagtttaccactccctatcagtgatagagaaaagtgaaagtcgagtttaccagtccctatcagtgatagagaaaagtgaaagtcgagtttaccactccctatcagtgatagagaaaagtgaaagtcgagtttaccactccctatcagtgatagagaaaagtgaaagtcgagctcgccatgggaggcgtggcctgggcgggactggggagtggcgagccctcagatcctgcatataagcagctgctttttgcctgtactgggtctctctggttagaccagatctgagcctgggagctctctggctaactagggaacccactgcttaagcctcaataaagcttgccttgagtgcttcaagtagtgtgtgcccgtctgttgtgtgactctggtaactagagatccctcagacccttttagtcagtgtggaaaatctctagcagtggcgcccgaacagggacttgaaagcgaaagggaaaccagaggagctctctcgacgcaggactcggcttgctgaagcgcgcacggcaagaggcgaggggcggcgactggtgagtacgccaaaaattttgactagcggaggctagaaggagagagatgggtgcgagagcgtcagtattaagcgggggagaattagatcgcgatgggaaaaaattcggttaaggccagggggaaagaaaaaatataaattaaaacatatagtatgggcaagcagggagctagaacgattcgcagttaatactggcctgttagaaacatcagaaggctgtagacaaatactgggacagctacaaccatcccttcagacaggatcagaagaacttagatcattatataatacagtagcaaccctctattgtgtgcatcaaaggatagagataaaagacaccaaggaagctttagacaagatagaggaagagcaaaacaaaagtaagaaaaaagcacagcaagcagcaggatcttcagacctggaaattccctacaatccccaaagtcaaggagtagtagaatctatgaataaagaattaaagaaaattataggacaggtaagagatcaggctgaacatcttaagacagcagtacaaatggcagtattcatccacaattttaaaagaaaaggggggattggggggtacagtgcaggggaaagaatagtagacataatagcaacagacatacaaactaaagaattacaaaaacaaattacaaaaattcaaaattttcgggtttattacagggacagcagaaatccactttggaaaggaccagcaaagctcctctggaaaggtgaaggggcagtagtaatacaagataatagtgacataaaagtagtgccaagaagaaaagcaaagatcattagggattatggaaaacagatggcaggtgatgattgtgtggcaagtagacaggatgaggattagaacatggaaaagtttagtaaaacaccataaggaggagatatgagggacaattggagaagtgaattatataaatataaagtagtaaaaattgaaccattaggagtagcacccaccaaggcaaagagaagagtggtgcagagagaaaaaagagcagtgggaataggagctttgttccttgggttcttgggagcagcaggaagcactatgggcgcagcgtcaatgacgctgacggtacaggccagacaattattgtctggtatagtgcagcagcagaacaatttgctgagggctattgaggcgcaacagcatctgttgcaactcacagtctggggcatcaagcagctccaggcaagaatcctggctgtggaaagatacctaaaggatcaacagctcctggggatttggggttgctctggaaaactcatttgcaccactgctgtgccttggaatgctagttggagtaataaatctctggaacagatttggaatcacacgacctggatggagtgggacagagaaattaacaattacacaagcttaatacactccttaattgaagaatcgcaaaaccagcaagaaaagaatgaacaagaattattggaattagataaatgggcaagtttgtggaattggtttaacataacaaattggctgtggtatataaaattattcataatgatagtaggaggcttggtaggtttaagaatagtttttgctgtactttctatagtgaatagagttaggcagggatattcaccattatcgtttcagacccacctcccaaccccgaggggaccgagctcaagcttcgaacgcgtgcggccgcatcgatgccgtagtacctttaagaccaatgacttacaaggcagctgtagatcttagccactttttaaaagaaaaggggggactggaagggctaattcactcccaaagaagacaagatccctgcaggcattcaaggccaggctggatgtggctctgggcagcctgggctgctggttgatgaccctgcacatagcagggggttggatctggatgagcactgtgctcctttgcaacccaggccgttctatgattctgtcattctaaatctctctttcagcctaaagctttttccccgtatccccccaggtgtctgcaggctcaaagagcagcgagaagcgttcagaggaaagcgatcccgtgccaccttccccgtgcccgggctgtccccgcacgctgccggctcggggatgcggggggagcgccggaccggagcggagccccgggcggctcgctgctgccccctagcgggggagggacgtaattacatccctgggggctttgggggggggctgtccccgtgagctccccagatctgctttttgcctgtactgggtctctctggttagaccagatctgagcctgggagctctctggctaactagggaacccactgcttaagcctcaataaagcttcagctgctcgagctagcagatctttttccctctgccaaaaattatggggacatcatgaagccccttgagcatctgacttctggctaataaaggaaatttattttcattgcaatagtgtgttggaattttttgtgtctctcactcggaaggacatatgggagggcaaatcatttaaaacatcagaatgagtatttggtttagagtttggcaacatatgcccatatgctggctgccatgaacaaaggttggctataaagaggtcatcagtatatgaaacagccccctgctgtccattccttattccatagaaaagccttgacttgaggttagattttttttatattttgttttgtgttatttttttctttaacatccctaaaattttccttacatgttttactagccagatttttcctcctctcctgactactcccagtcatagctgtccctcttctcttatggagatccctcgacctgcagcccaagcttggcgtaatcatggtcatagctgtttcctgtgtgaaattgttatccgctcacaattccacacaacatacgagccggaagcataaagtgtaaagcctggggtgcctaatgagtgagctaactcacattaattgcgttgcgctcactgcccgctttccagtcgggaaacctgtcgtgccagcggatccgcatctcaattagtcagcaaccatagtcccgcccctaactccgcccatcccgcccctaactccgcccagttccgcccattctccgccccatggctgactaattttttttatttatgcagaggccgaggccgcctcggcctctgagctattccagaagtagtgaggaggcttttttggaggcctaggcttttgcaaaaagctgtcgactgcagaggcctgcatgcaagcttggcgtaatcatggtcatagctgtttcctgtgtgaaattgttatccgctcacaattccacacaacatacgagccggaagcataaagtgtaaagcctggggtgcctaatgagtgagctaactcacattaattgcgttgcgctcactgcccgctttccagtcgggaaacctgtcgtgccagctgcattaatgaatcggccaacgcgcggggagaggcggtttgcgtattgggcgctcttccgcttcctcgctcactgactcgctgcgctcggtcgttcggctgcggcgagcggtatcagctcactcaaaggcggtaatacggttatccacagaatcaggggataacgcaggaaagaacatgtgagcaaaaggccagcaaaaggccaggaaccgtaaaaaggccgcgttgctggcgtttttccataggctccgcccccctgacgagcatcacaaaaatcgacgctcaagtcagaggtggcgaaacccgacaggactataaagataccaggcgtttccccctggaagctccctcgtgcgctctcctgttccgaccctgccgcttaccggatacctgtccgcctttctcccttcgggaagcgtggcgctttctcatagctcacgctgtaggtatctcagttcggtgtaggtcgttcgctccaagctgggctgtgtgcacgaaccccccgttcagcccgaccgctgcgccttatccggtaactatcgtcttgagtccaacccggtaagacacgacttatcgccactggcagcagccactggtaacaggattagcagagcgaggtatgtaggcggtgctacagagttcttgaagtggtggcctaactacggctacactagaagaacagtatttggtatctgcgctctgctgaagccagttaccttcggaaaaagagttggtagctcttgatccggcaaacaaaccaccgctggtagcggtggtttttttgtttgcaagcagcagattacgcgcagaaaaaaaggatctcaagaagatcctttgatcttttctacggggtctgacgctcagtggaacgaaaactcacgttaagggattttggtcatgagattatcaaaaaggatcttcacctagatccttttaaattaaaaatgaagttttaaatcaatctaaagtatatatgagtaaacttggtctgacagttaccaatgcttaatcagtgaggcacctatctcagcgatctgtctatttcgttcatccatagttgcctgactccccgtcgtgtagataactacgatacgggagggcttaccatctggccccagtgctgcaatgataccgcgagacccacgctcaccggctccagatttatcagcaataaaccagccagccggaagggccgagcgcagaagtggtcctgcaactttatccgcctccatccagtctattaattgttgccgggaagctagagtaagtagttcgccagttaatagtttgcgcaacgttgttgccattgctacaggcatcgtggtgtcacgctcgtcgtttggtatggcttcattcagctccggttcccaacgatcaaggcgagttacatgatcccccatgttgtgcaaaaaagcggttagctccttcggtcctccgatcgttgtcagaagtaagttggccgcagtgttatcactcatggttatggcagcactgcataattctcttactgtcatgccatccgtaagatgcttttctgtgactggtgagtactcaaccaagtcattctgagaatagtgtatgcggcgaccgagttgctcttgcccggcgtcaatacgggataataccgcgccacatagcagaactttaaaagtgctcatcattggaaaacgttcttcggggcgaaaactctcaaggatcttaccgctgttgagatccagttcgatgtaacccactcgtgcacccaactgatcttcagcatcttttactttcaccagcgtttctgggtgagcaaaaacaggaaggcaaaatgccgcaaaaaagggaataagggcgacacggaaatgttgaatactcatactcttcctttttcaatattattgaagcatttatcagggttattgtctcatgagcggatacatatttgaatgtatttagaaaaataaacaaataggggttccgcgcacatttccccgaaaagtgccacctgacgtctaagaaaccattattatcatgacattaacctataaaaataggcgtatcacgaggccctttcgtctcgcgcgtttcggtgatgacggtgaaaacctctgacacatgcagctcccggagacggtcacagcttgtctgtaagcggatgccgggagcagacaagcccgtcagggcgcgtcagcgggtgttggcgggtgtcggggctggcttaactatgcggcatcagagcagattgtactgagagtgcaccatatgcggtgtgaaataccgcacagatgcgtaaggagaaaataccgcatcaggcgccattcgccattcaggctgcgcaactgttgggaagggcgatcggtgcgggcctcttcgctattacgccagctggcgaaagggggatgtgctgcaaggcgattaagttgggtaacgccagggttttcccagtcacgacgttgtaaaacgacggccagtgaattc

SEQ ID NO: 2 - DNA, 3901 bp, Artificial Sequence
  Synthetic: TL20C vector backbone
ggccgcctcggccaaacagcccttgagtttaccactccctatcagtgatagagaaaagtgaaagtcgagtttaccactccctatcagtgatagagaaaagtgaaagtcgagtttaccactccctatcagtgatagagaaaagtgaaagtcgagtttaccactccctatcagtgatagagaaaagtgaaagtcgagtttaccagtccctatcagtgatagagaaaagtgaaagtcgagtttaccactccctatcagtgatagagaaaagtgaaagtcgagtttaccactccctatcagtgatagagaaaagtgaaagtcgagctcgccatgggaggcgtggcctgggcgggactggggagtggcgagccctcagatcctgcatataagcagctgctttttgcctgtactgggtctctctggttagaccagatctgagcctgggagctctctggctaactagggaacccactgcttaagcctcaataaagcttgccttgagtgcttcaagtagtgtgtgcccgtctgttgtgtgactctggtaactagagatccctcagacccttttagtcagtgtggaaaatctctagcagtggcgcccgaacagggacttgaaagcgaaagggaaaccagaggagctctctcgacgcaggactcggcttgctgaagcgcgcacggcaagaggcgaggggcggcgactggtgagtacgccaaaaattttgactagcggaggctagaaggagagagatgggtgcgagagcgtcagtattaagcgggggagaattagatcgcgatgggaaaaaattcggttaaggccagggggaaagaaaaaatataaattaaaacatatagtatgggcaagcagggagctagaacgattcgcagttaatactggcctgttagaaacatcagaaggctgtagacaaatactgggacagctacaaccatcccttcagacaggatcagaagaacttagatcattatataatacagtagcaaccctctattgtgtgcatcaaaggatagagataaaagacaccaaggaagctttagacaagatagaggaagagcaaaacaaaagtaagaaaaaagcacagcaagcagcaggatcttcagacctggaaattccctacaatccccaaagtcaaggagtagtagaatctatgaataaagaattaaagaaaattataggacaggtaagagatcaggctgaacatcttaagacagcagtacaaatggcagtattcatccacaattttaaaagaaaaggggggattggggggtacagtgcaggggaaagaatagtagacataatagcaacagacatacaaactaaagaattacaaaaacaaattacaaaaattcaaaattttcgggtttattacagggacagcagaaatccactttggaaaggaccagcaaagctcctctggaaaggtgaaggggcagtagtaatacaagataatagtgacataaaagtagtgccaagaagaaaagcaaagatcattagggattatggaaaacagatggcaggtgatgattgtgtggcaagtagacaggatgaggattagaacatggaaaagtttagtaaaacaccataaggaggagatatgagggacaattggagaagtgaattatataaatataaagtagtaaaaattgaaccattaggagtagcacccaccaaggcaaagagaagagtggtgcagagagaaaaaagagcagtgggaataggagctttgttccttgggttcttgggagcagcaggaagcactatgggcgcagcgtcaatgacgctgacggtacaggccagacaattattgtctggtatagtgcagcagcagaacaatttgctgagggctattgaggcgcaacagcatctgttgcaactcacagtctggggcatcaagcagctccaggcaagaatcctggctgtggaaagatacctaaaggatcaacagctcctggggatttggggttgctctggaaaactcatttgcaccactgctgtgccttggaatgctagttggagtaataaatctctggaacagatttggaatcacacgacctggatggagtgggacagagaaattaacaattacacaagcttaatacactccttaattgaagaatcgcaaaaccagcaagaaaagaatgaacaagaattattggaattagataaatgggcaagtttgtggaattggtttaacataacaaattggctgtggtatataaaattattcataatgatagtaggaggcttggtaggtttaagaatagtttttgctgtactttctatagtgaatagagttaggcagggatattcaccattatcgtttcagacccacctcccaaccccgaggggaccgagctcaagcttcgaacgcgtgcggccgcatcgatgccgtagtacctttaagaccaatgacttacaaggcagctgtagatcttagccactttttaaaagaaaaggggggactggaagggctaattcactcccaaagaagacaagatccctgcaggcattcaaggccaggctggatgtggctctgggcagcctgggctgctggttgatgaccctgcacatagcagggggttggatctggatgagcactgtgctcctttgcaacccaggccgttctatgattctgtcattctaaatctctctttcagcctaaagctttttccccgtatccccccaggtgtctgcaggctcaaagagcagcgagaagcgttcagaggaaagcgatcccgtgccaccttccccgtgcccgggctgtccccgcacgctgccggctcggggatgcggggggagcgccggaccggagcggagccccgggcggctcgctgctgccccctagcgggggagggacgtaattacatccctgggggctttgggggggggctgtccccgtgagctccccagatctgctttttgcctgtactgggtctctctggttagaccagatctgagcctgggagctctctggctaactagggaacccactgcttaagcctcaataaagcttcagctgctcgagctagcagatctttttccctctgccaaaaattatggggacatcatgaagccccttgagcatctgacttctggctaataaaggaaatttattttcattgcaatagtgtgttggaattttttgtgtctctcactcggaaggacatatgggagggcaaatcatttaaaacatcagaatgagtatttggtttagagtttggcaacatatgcccatatgctggctgccatgaacaaaggttggctataaagaggtcatcagtatatgaaacagccccctgctgtccattccttattccatagaaaagccttgacttgaggttagattttttttatattttgttttgtgttatttttttctttaacatccctaaaattttccttacatgttttactagccagatttttcctcctctcctgactactcccagtcatagctgtccctcttctcttatggagatccctcgacctgcagcccaagcttggcgtaatcatggtcatagctgtttcctgtgtgaaattgttatccgctcacaattccacacaacatacgagccggaagcataaagtgtaaagcctggggtgcctaatgagtgagctaactcacattaattgcgttgcgctcactgcccgctttccagtcgggaaacctgtcgtgccagcggatccgcatctcaattagtcagcaaccatagtcccgcccctaactccgcccatcccgcccctaactccgcccagttccgcccattctccgccccatggctgactaattttttttatttatgcagaggccgaggccgcctcggcctctgagctattccagaagtagtgaggaggcttttttggaggcctaggcttttgcaaaaagct

SEQ ID NO: 3 - DNA, 343 bp, Artificial Sequence
  Synthetic: nucleotide sequence encoding the packing signal
agtattaagcgggggagaattagatcgcgatgggaaaaaattcggttaaggccagggggaaagaaaaaatataaattaaaacatatagtatgggcaagcagggagctagaacgattcgcagttaatactggcctgttagaaacatcagaaggctgtagacaaatactgggacagctacaaccatcccttcagacaggatcagaagaacttagatcattatataatacagtagcaaccctctattgtgtgcatcaaaggatagagataaaagacaccaaggaagctttagacaagatagaggaagagcaaaacaaaagtaagaaaaaagcacagcaagcagcag

SEQ ID NO: 4 - DNA, 477 bp, Artificial Sequence
  Synthetic: Central polypurine tract (cppt)
aattccctacaatccccaaagtcaaggagtagtagaatctatgaataaagaattaaagaaaattataggacaggtaagagatcaggctgaacatcttaagacagcagtacaaatggcagtattcatccacaattttaaaagaaaaggggggattggggggtacagtgcaggggaaagaatagtagacataatagcaacagacatacaaactaaagaattacaaaaacaaattacaaaaattcaaaattttcgggtttattacagggacagcagaaatccactttggaaaggaccagcaaagctcctctggaaaggtgaaggggcagtagtaatacaagataatagtgacataaaagtagtgccaagaagaaaagcaaagatcattagggattatggaaaacagatggcaggtgatgattgtgtggcaagtagacaggatgaggattagaacatggaaaagtttagtaaaacaccata

SEQ ID NO: 5 - DNA, 769 bp, Artificial Sequence
  Synthetic: nucleotide sequence encoding the rev response element
aggaggagatatgagggacaattggagaagtgaattatataaatataaagtagtaaaaattgaaccattaggagtagcacccaccaaggcaaagagaagagtggtgcagagagaaaaaagagcagtgggaataggagctttgttccttgggttcttgggagcagcaggaagcactatgggcgcagcgtcaatgacgctgacggtacaggccagacaattattgtctggtatagtgcagcagcagaacaatttgctgagggctattgaggcgcaacagcatctgttgcaactcacagtctggggcatcaagcagctccaggcaagaatcctggctgtggaaagatacctaaaggatcaacagctcctggggatttggggttgctctggaaaactcatttgcaccactgctgtgccttggaatgctagttggagtaataaatctctggaacagatttggaatcacacgacctggatggagtgggacagagaaattaacaattacacaagcttaatacactccttaattgaagaatcgcaaaaccagcaagaaaagaatgaacaagaattattggaattagataaatgggcaagtttgtggaattggtttaacataacaaattggctgtggtatataaaattattcataatgatagtaggaggcttggtaggtttaagaatagtttttgctgtactttctatagtgaatagagttaggcagggatattcaccattatcgtttcagacccacctcccaaccccgaggggaccg

SEQ ID NO: 6 - DNA, 181 bp, Artificial Sequence
  Synthetic: nucleotide sequence encoding the self-inactivating long terminal repeat
gggtctctctggttagaccagatctgagcctgggagctctctggctaactagggaacccactgcttaagcctcaataaagcttgccttgagtgcttcaagtagtgtgtgcccgtctgttgtgtgactctggtaactagagatccctcagacccttttagtcagtgtggaaaatctctagca

SEQ ID NO: 7 - DNA, 25 bp, Artificial Sequence
  Synthetic: nucleotide sequence encoding the multiple cloning site
ttcgaacgcgtgcggccgcatcgat

SEQ ID NO: 8 - DNA, 1978 bp, Artificial Sequence
  Synthetic: LVSH5/C46
gaacgctgacgtcatcaacccgctccaaggaatcgcgggcccagtgtcactaggcgggaacacccagcgcgcgtgcgccctggcaggaagatggctgtgagggacaggggagtggcgccctgcaatatttgcatgtcgctatgtgttctgggaaatcaccataaacgtgaaatgtctttggatttgggaatcttataagttctgtatgagaccacggatccccgagcaagctcagtttacaccttgtccgacggtgtaaactgagcttgctctttttgagacgagtcctcgagccataaagatggttaattaacccacccaagatctggcctccgcgccgggttttggcgcctcccgcgggcgcccccctcctcacggcgagcgctgccacgtcagacgaagggcgcagcgagcgtcctgatccttccgcccggacgctcaggacagcggcccgctgctcataagactcggccttagaaccccagtatcagcagaaggacattttaggacgggacttgggtgactctagggcactggttttctttccagagagcggaacaggcgaggaaaagtagtcccttctcggcgattctgcggagggatctccgtggggcggtgaacgccgatgattatataaggacgcgccgggtgtggcacagctagttccgtcgcagccgggatttgggtcgcggttcttgtttgtggatcgctgtgatcgtcacttggtgagtagcgggctgctgggctggccggggctttcgtggccgccgggccgctcggtgggacggaagcgtgtggagagaccgccaagggctgtagtctgggtccgcgagcaaggttgccctgaactgggggttggggggagcgcagcaaaatggcggctgttcccgagtcttgaatggaagacgcttgtgaggcgggctgtgaggtcgttgaaacaaggtggggggcatggtgggcggcaagaacccaaggtcttgaggccttcgctaatgcgggaaagctcttattcgggtgagatgggctggggcaccatctggggaccctgacgtgaagtttgtcactgactggagaactcggtttgtcgtctgttgcgggggcggcagttatggcggtgccgttgggcagtgcacccgtacctttgggagcgcgcgccctcgtcgtgtcgtgacgtcacccgttctgttggcttataatgcagggtggggccacctgccggtaggtgtgcggtaggcttttctccgtcgcaggacgcagggttcgggcctagggtaggctctcctgaatcgacaggcgccggacctctggtgaggggagggataagtgaggcgtcagtttctttggtcggttttatgtacctatcttcttaagtagctgaagctccggttttgaactatgcgctcggggttggcgagtgtgttttgtgaagttttttaggcaccttttgaaatgtaatcatttgggtcaatatgtaattttcagtgttagactagtaaattgtccgctaaattctggccgtttttggcttttttgttagacgaagcttggtaccgagctcggatccgccaccatgggagcaggagcaaccggaagggcaatggacggaccaagattgttacttctgctcctgctaggcgtgagcctgggaggagcaaggagctggatggagtgggacagggagatcaacaactacaccagcctgatccacagcctgatcgaggagagccagaaccagcaggagaagaacgagcaggagctgctggagctggacaagtgggccagcctgtggaactggttccggagcgagcggaagtgctgcgtggagtgcccaccatgcccagcaccaccagtggcaggacccctgatcgcactggtgaccagcggagccctgctggccgtgctgggcatcacaggctacttcctgatgaacaggaggagctggagcccaaccggagagcggctggagctggagccatga

SEQ ID NO: 9 - DNA, 1113 bp, Artificial Sequence
  Synthetic: PGK-BLE SEQUENCE
ccagcctttggaattcctgcaggatgggattctaccgggtaggggaggcgcttttcccaaggcagtctggagcatgcgctttagcagccccgctgggcacttggcgctacacaagtggcctctggcctcgcacacattccacatccaccggtaggcgccaaccggctccgttctttggtggccccttcgcgccaccttctactcctcccctagtcaggaagttcccccccgccccgcagctcgcgtcgtgcaggacgtgacaaatggaagtagcacgtctcactagtctcgtgcagatggacagcaccgctgagcaatggaagcgggtaggcctttggggcagcggccaatagcagctttgctccttcgctttctgggctcaggggcggggcgggcgcccgaaggtcctccggaggcccggcattctgcacgcttcaaaagcgcacgtctgccgcgctgttctcctcttcctcatctccgggcctttcgacctggatcctgcagcacgtgttgacaattaatcatcggcatagtatatcggcatagtataatacgactcactataggagggccaccatggccaagttgaccagtgccgttccggtgctcaccgcgcgcgacgtcgccggagcggtcgagttctggaccgaccggctcgggttctcccgggacttcgtggaggacgacttcgccggtgtggtccgggacgacgtgaccctgttcatcagcgcggtccaggaccaggtggtgccggacaacaccctggcctgggtgtgggtgcgcggcctggacgagctgtacgccgagtggtcggaggtcgtgtccacgaacttccgggacgcctccgggccggccatgaccgagatcggcgagcagccgtgggggcgggagttcgccctgcgcgacccggccggcaactgcgtgcacttcgtggccgaggagcaggactgatgctttatttgtgaaatttgtgatgctattgctttatttgtaaccattataagctgcaataaacaagttaacaacaacaattgcattcattttatgtttcaggttcagggggaggtgtgggaggttttttaaactagtgagtcgtattacccagcctttggg

SEQ ID NO: 10 - DNA, 288 bp, Artificial Sequence
  Synthetic: (7tetO): doxycycline repressible promoter
tttaccactccctatcagtgatagagaaaagtgaaagtcgagtttaccactccctatcagtgatagagaaaagtgaaagtcgagtttaccactccctatcagtgatagagaaaagtgaaagtcgagtttaccactccctatcagtgatagagaaaagtgaaagtcgagtttaccagtccctatcagtgatagagaaaagtgaaagtcgagtttaccactccctatcagtgatagagaaaagtgaaagtcgagtttaccactccctatcagtgatagagaaaagtgaaa

SEQ ID NO: 11 - DNA, 98 bp, Artificial Sequence
  Synthetic: HIV LTR R5 region
gggtctctctggttagaccagatctgagcctgggagctctctggctaactagggaacccactgcttaagcctcaataaagcttgccttgagtgcttca

SEQ ID NO: 12 - DNA, 83 bp, Artificial Sequence
  Synthetic: HIV LTR U5 region
agtagtgtgtgcccgtctgttgtgtgactctggtaactagagatccctcagacccttttagtcagtgtggaaaatctctagca

SEQ ID NO: 13 - DNA, 412 bp, Artificial Sequence
  Synthetic: chicken HS4 400 bp chromatin insulator
atccctgcaggcattcaaggccaggctggatgtggctctgggcagcctgggctgctggttgatgaccctgcacatagcagggggttggatctggatgagcactgtgctcctttgcaacccaggccgttctatgattctgtcattctaaatctctctttcagcctaaagctttttccccgtatccccccaggtgtctgcaggctcaaagagcagcgagaagcgttcagaggaaagcgatcccgtgccaccttccccgtgcccgggctgtccccgcacgctgccggctcggggatgcggggggagcgccggaccggagcggagccccgggcggctcgctgctgccccctagcgggggagggacgtaattacatccctgggggctttgggggggggctgtccccgtgagctcccc

SEQ ID NO: 14 - DNA, 449 bp, Artificial Sequence
  Synthetic: rabbit beta-globin polyadenylation signal
gatctttttccctctgccaaaaattatggggacatcatgaagccccttgagcatctgacttctggctaataaaggaaatttattttcattgcaatagtgtgttggaattttttgtgtctctcactcggaaggacatatgggagggcaaatcatttaaaacatcagaatgagtatttggtttagagtttggcaacatatgcccatatgctggctgccatgaacaaaggttggctataaagaggtcatcagtatatgaaacagccccctgctgtccattccttattccatagaaaagccttgacttgaggttagattttttttatattttgttttgtgttatttttttctttaacatccctaaaattttccttacatgttttactagccagatttttcctcctctcctgactactcccagtcatagctgtccctcttctcttatggagatc

SEQ ID NO: 15 - DNA, 2664 bp, Artificial Sequence
  Synthetic: pUC57 Plasmid portion
gtcgactgcagaggcctgcatgcaagcttggcgtaatcatggtcatagctgtttcctgtgtgaaattgttatccgctcacaattccacacaacatacgagccggaagcataaagtgtaaagcctggggtgcctaatgagtgagctaactcacattaattgcgttgcgctcactgcccgctttccagtcgggaaacctgtcgtgccagctgcattaatgaatcggccaacgcgcggggagaggcggtttgcgtattgggcgctcttccgcttcctcgctcactgactcgctgcgctcggtcgttcggctgcggcgagcggtatcagctcactcaaaggcggtaatacggttatccacagaatcaggggataacgcaggaaagaacatgtgagcaaaaggccagcaaaaggccaggaaccgtaaaaaggccgcgttgctggcgtttttccataggctccgcccccctgacgagcatcacaaaaatcgacgctcaagtcagaggtggcgaaacccgacaggactataaagataccaggcgtttccccctggaagctccctcgtgcgctctcctgttccgaccctgccgcttaccggatacctgtccgcctttctcccttcgggaagcgtggcgctttctcatagctcacgctgtaggtatctcagttcggtgtaggtcgttcgctccaagctgggctgtgtgcacgaaccccccgttcagcccgaccgctgcgccttatccggtaactatcgtcttgagtccaacccggtaagacacgacttatcgccactggcagcagccactggtaacaggattagcagagcgaggtatgtaggcggtgctacagagttcttgaagtggtggcctaactacggctacactagaagaacagtatttggtatctgcgctctgctgaagccagttaccttcggaaaaagagttggtagctcttgatccggcaaacaaaccaccgctggtagcggtggtttttttgtttgcaagcagcagattacgcgcagaaaaaaaggatctcaagaagatcctttgatcttttctacggggtctgacgctcagtggaacgaaaactcacgttaagggattttggtcatgagattatcaaaaaggatcttcacctagatccttttaaattaaaaatgaagttttaaatcaatctaaagtatatatgagtaaacttggtctgacagttaccaatgcttaatcagtgaggcacctatctcagcgatctgtctatttcgttcatccatagttgcctgactccccgtcgtgtagataactacgatacgggagggcttaccatctggccccagtgctgcaatgataccgcgagacccacgctcaccggctccagatttatcagcaataaaccagccagccggaagggccgagcgcagaagtggtcctgcaactttatccgcctccatccagtctattaattgttgccgggaagctagagtaagtagttcgccagttaatagtttgcgcaacgttgttgccattgctacaggcatcgtggtgtcacgctcgtcgtttggtatggcttcattcagctccggttcccaacgatcaaggcgagttacatgatcccccatgttgtgcaaaaaagcggttagctccttcggtcctccgatcgttgtcagaagtaagttggccgcagtgttatcactcatggttatggcagcactgcataattctcttactgtcatgccatccgtaagatgcttttctgtgactggtgagtactcaaccaagtcattctgagaatagtgtatgcggcgaccgagttgctcttgcccggcgtcaatacgggataataccgcgccacatagcagaactttaaaagtgctcatcattggaaaacgttcttcggggcgaaaactctcaaggatcttaccgctgttgagatccagttcgatgtaacccactcgtgcacccaactgatcttcagcatcttttactttcaccagcgtttctgggtgagcaaaaacaggaaggcaaaatgccgcaaaaaagggaataagggcgacacggaaatgttgaatactcatactcttcctttttcaatattattgaagcatttatcagggttattgtctcatgagcggatacatatttgaatgtatttagaaaaataaacaaataggggttccgcgcacatttccccgaaaagtgccacctgacgtctaagaaaccattattatcatgacattaacctataaaaataggcgtatcacgaggccctttcgtctcgcgcgtttcggtgatgacggtgaaaacctctgacacatgcagctcccggagacggtcacagcttgtctgtaagcggatgccgggagcagacaagcccgtcagggcgcgtcagcgggtgttggcgggtgtcggggctggcttaactatgcggcatcagagcagattgtactgagagtgcaccatatgcggtgtgaaataccgcacagatgcgtaaggagaaaataccgcatcaggcgccattcgccattcaggctgcgcaactgttgggaagggcgatcggtgcgggcctcttcgctattacgccagctggcgaaagggggatgtgctgcaaggcgattaagttgggtaacgccagggttttcccagtcacgacgttgtaaaacgacggccagtgaattc